European Patent Application EP 4 349 372 A1, published April 10, 2024. Title: Antibody drug conjugate, and preparation method therefor and use thereof. Applicant: SICHUAN KELUN-BIOTECH BIOPHARMACEUTICAL CO., LTD. KLUS PHARMA INC. The sequence listing filed with the application follows.

SEQUENCE LISTING (48 sequences)

SEQ ID NO: 1 - protein, 118 aa, artificial
  19F6_Hu35V1 VH
QVQLQESGPGLVKPSQTLSLTCTVSGYSITSDYAWNWIRQFPGKGLEWIGYISYSGSIRYNPSLKSRVTISRDTSKNQFSLKLSSVTAADTAVYYCARGEITYYFDYWGQGTLVTVSS

SEQ ID NO: 2 - protein, 107 aa, artificial
  19F6_Hu35V1 VL
ETTLTQSPAFMSATPGDKVTISCKASTSIDDDMNWYQQKPGEPPKLIISEGNTLRPGIPPRFSSSGYGTDFTFTINKIKSEDAATYYCLQSNDLPLTFGQGTKLEIK

SEQ ID NO: 3 - protein, 8 aa, artificial
  19F6_Hu35V1 Chothia CDR-H1
GYSITSDY

SEQ ID NO: 4 - protein, 5 aa, artificial
  19F6_Hu35V1 Chothia CDR-H2
SYSGS

SEQ ID NO: 5 - protein, 9 aa, artificial
  19F6_Hu35V1 Chothia/AbM/Kabat CDR-H3
GEITYYFDY

SEQ ID NO: 6 - protein, 11 aa, artificial
  19F6_Hu35V1 AbM/Kabat/Chothia CDR-L1
KASTSIDDDMN

SEQ ID NO: 7 - protein, 7 aa, artificial
  19F6_Hu35V1 AbM/Kabat/Chothia CDR-L2
EGNTLRP

SEQ ID NO: 8 - protein, 9 aa, artificial
  19F6_Hu35V1 AbM/Kabat/Chothia /IMGT CDR-L3
LQSNDLPLT

SEQ ID NO: 9 - protein, 121 aa, artificial
  3D8_HuC24 VH
EVQLVESGGGLVQPGGSLRLSCAASGFTFSSYAMSWVRQAPGKGLEWVASINSGGSTYYPDSVKGRFTISRDNAKNSLYLQMNSLRAEDTAVYYCARVNYYGYGDYAMDYWGQGTLVTVSS

SEQ ID NO: 10 - protein, 107 aa, artificial
  3D8_HuC24 VL
DIQMTQSPSSLSASVGDRVTITCQASQDISNYLTWFQQKPGKSPKTLIHRANRLVTGVPSRFSGSGSGTDFTFTISSLQPEDIATYYCLQYDEFPYTFGGGTKVEIK

SEQ ID NO: 11 - protein, 7 aa, artificial
  3D8_HuC24 Chothia CDR-H1
GFTFSSY

SEQ ID NO: 12 - protein, 5 aa, artificial
  3D8_HuC24 Chothia CDR-H2
NSGGS

SEQ ID NO: 13 - protein, 13 aa, artificial
  3D8_HuC24 AbM/Kabat/Chothia CDR-H3
VNYYGYGDYAMDY

SEQ ID NO: 14 - protein, 11 aa, artificial
  3D8_HuC24/38F8_Hu57 AbM/Kabat/Chothia CDR-L1
QASQDISNYLT

SEQ ID NO: 15 - protein, 7 aa, artificial
  3D8_HuC24/38F8_Hu57 AbM/Kabat/Chothia CDR-L2
RANRLVT

SEQ ID NO: 16 - protein, 9 aa, artificial
  3D8_HuC24/38F8_Hu57 IMGT/Abm/Kabat/Chothia CDR-L3
LQYDEFPYT

SEQ ID NO: 17 - protein, 120 aa, artificial
  38F8_Hu57 VH
EVQLVESGGGLVQPGGSLRLSCAASGFTFSNYAMSWVRQAPEKRLEWVASISSGGPTYYPDSVKGRFTVSRDNSKNTLYLQMNSLRAEDTAVYYCARGYRYDVNWYFDVWGAGTMVTVSS

SEQ ID NO: 18 - protein, 107 aa, artificial
  38F8_Hu57 VL
DIQMTQSPSSLSASVGDRVTITCQASQDISNYLTWFQQKPGKSPKTLIHRANRLVTGVPSRFSGSGSGTDYTFTISSLQPEDIAIYYCLQYDEFPYTFGGGTKVEIK

SEQ ID NO: 19 - protein, 7 aa, artificial
  38F8_Hu57 Chothia CDR-H1
GFTFSNY

SEQ ID NO: 20 - protein, 5 aa, artificial
  38F8_Hu57 Chothia CDR-H2
SSGGP

SEQ ID NO: 21 - protein, 12 aa, artificial
  38F8_Hu57 AbM/Kabat/Chothia CDR-H3
GYRYDVNWYFDV

SEQ ID NO: 22 - protein, 330 aa, artificial [sequence omitted]

SEQ ID NO: 23 - protein, 107 aa, artificial [sequence omitted]

SEQ ID NO: 24 - protein, 9 aa, artificial
  19F6_Hu35V1 IMGT CDR-H1
GYSITSDYA

SEQ ID NO: 25 - protein, 7 aa, artificial
  19F6_Hu35V1 IMGT CDR-H2
ISYSGSI

SEQ ID NO: 26 - protein, 11 aa, artificial
  19F6_Hu35V1 IMGT CDR-H3
ARGEITYYFDY

SEQ ID NO: 27 - protein, 6 aa, artificial
  19F6_Hu35V1 IMGT CDR-L1
TSIDDD

SEQ ID NO: 28 - protein, 3 aa, artificial
  19F6_Hu35V1 IMGT CDR-L2
EGN

SEQ ID NO: 29 - protein, 11 aa, artificial
  19F6_Hu35V1 AbM CDR-H1
GYSITSDYAWN

SEQ ID NO: 30 - protein, 9 aa, artificial
  19F6_Hu35V1 AbM CDR-H2
YISYSGSIR

SEQ ID NO: 31 - protein, 6 aa, artificial
  19F6_Hu35V1 Kabat CDR-H1
SDYAWN

SEQ ID NO: 32 - protein, 16 aa, artificial
  19F6_Hu35V1 Kabat CDR-H2
YISYSGSIRYNPSLKS

SEQ ID NO: 33 - protein, 8 aa, artificial
  3D8_HuC24 IMGT CDR-H1
GFTFSSYA

SEQ ID NO: 34 - protein, 7 aa, artificial
  3D8_HuC24 IMGT CDR-H2
INSGGST

SEQ ID NO: 35 - protein, 15 aa, artificial
  3D8_HuC24 IMGT CDR-H3
ARVNYYGYGDYAMDY

SEQ ID NO: 36 - protein, 10 aa, artificial
  3D8_HuC24 AbM CDR-H1
GFTFSSYAMS

SEQ ID NO: 37 - protein, 9 aa, artificial
  3D8_HuC24 AbM CDR-H2
SINSGGSTY

SEQ ID NO: 38 - protein, 5 aa, artificial
  3D8_HuC24 Kabat CDR-H1
SYAMS

SEQ ID NO: 39 - protein, 16 aa, artificial
  3D8_HuC24 Kabat CDR-H2
SINSGGSTYYPDSVKG

SEQ ID NO: 40 - protein, 8 aa, artificial
  38F8_Hu57 IMGT CDR-H1
GFTFSNYA

SEQ ID NO: 41 - protein, 7 aa, artificial
  38F8_Hu57 IMGT CDR-H2
ISSGGPT

SEQ ID NO: 42 - protein, 14 aa, artificial
  38F8_Hu57 IMGT CDR-H3
ARGYRYDVNWYFDV

SEQ ID NO: 43 - protein, 6 aa, artificial
  38F8_Hu57 /3D8_HuC24 IMGT CDR-L1
QDISNY

SEQ ID NO: 44 - protein, 3 aa, artificial
  38F8_Hu57/3D8_HuC24 IMGT CDR-L2
RAN

SEQ ID NO: 45 - protein, 10 aa, artificial
  38F8_Hu57 AbM  CDR-H1
GFTFSNYAMS

SEQ ID NO: 46 - protein, 9 aa, artificial
  38F8_Hu57 AbM  CDR-H2
SISSGGPTY

SEQ ID NO: 47 - protein, 5 aa, artificial
  38F8_Hu57 Kabat CDR-H1
NYAMS

SEQ ID NO: 48 - protein, 16 aa, artificial
  38F8_Hu57 Kabat CDR-H2
SISSGGPTYYPDSVKG